European Patent Application EP 4 814 119 A1, published September 30, 2026. Title: A microorganism of Corynebacterium genus having enhanced L-amino acid productivity and a method for producing L-amino acid using the same. Applicant: DAESANG CORPORATION. The sequence listing filed with the application follows.

SEQUENCE LISTING (44 sequences)

SEQ ID NO: 1 - DNA, 1149 bp, Corynebacterium glutamicum
  source 1..1149: mol_type = genomic DNA
ttgcgagataactggccgtgtgatactcgaatggacaatggcatgacaatcaccacagaacattcaactcatcctgatcttgatttcaatgatgagatttatcgggaactaaaccgcatctgcgcttcgctatctcaacagtgcagcacatatcaaccagagttccgtacctgcctagatgctgctttccaagctttgcgaggtggcaagttaatccgccctcgaatgctactggggctatacaacacgcttgtagacgatgacattgaggtcaaactcaacaccgttttacaggtagcagtggctttagaactactgcatttttcccttttggttcatgacgatgttattgacggagacctctatcgccgaggcaaacttaattttattgggcagattctcatgcatcgcacacctgaaagttttgcacaaatccagcgcgatccagagcatctagattgggcacaatctaatggactgcttatgggaaatctttttcttgctgccacccatcaaatcttcgcgcgccttgaccttccacatcaccaacgggttcgacttttagatttactcaaccacacgataaatgacactattgtgggtgagtttcttgatgtgggattaagcagcaaagccatcagccccaatatggacattgctctagaaatgagtcggctaaaaacagccacatacacttttgaacttccaatgagagcagcggcaattctcgcggaactacctcaggagattgaaacaaagataggtgagataggcacaaacttgggcatcgcttatcaattgcaggacgattacttatctacttttggtgacgcagccgaacacggcaaagatgccttttctgaccttcgagaaggaaaagaaactacaattatcgccttcgctcgagatactgctaaatggactgatattcaagacaacttcggctccgcagatctgagcacctctcaggcagagcgaattcaacatcttctcatacagtgtggagcaaagaatcactccttgaatgccatctccgaccacttaaatatctgccgttcgatgatcaaaacactaagcccccaggtagatcccaaggctcaaaatttattacttaaacaagttgagcaactagccagccgcaaatcttag

SEQ ID NO: 2 - protein, 382 aa, Corynebacterium glutamicum
MRDNWPCDTRMDNGMTITTEHSTHPDLDFNDEIYRELNRICASLSQQCSTYQPEFRTCLDAAFQALRGGKLIRPRMLLGLYNTLVDDDIEVKLNTVLQVAVALELLHFSLLVHDDVIDGDLYRRGKLNFIGQILMHRTPESFAQIQRDPEHLDWAQSNGLLMGNLFLAATHQIFARLDLPHHQRVRLLDLLNHTINDTIVGEFLDVGLSSKAISPNMDIALEMSRLKTATYTFELPMRAAAILAELPQEIETKIGEIGTNLGIAYQLQDDYLSTFGDAAEHGKDAFSDLREGKETTIIAFARDTAKWTDIQDNFGSADLSTSQAERIQHLLIQCGAKNHSLNAISDHLNICRSMIKTLSPQVDPKAQNLLLKQVEQLASRKS

SEQ ID NO: 3 - DNA, 915 bp, Corynebacterium glutamicum
  source 1..915: mol_type = genomic DNA
atgacacaccaaaattcgcctctcttccttaaaagtgcactgagactttacaatcgggcctcattcaaggcttcacataaagtgatcgaagaatattcgacgagcttcagtctgtctacgtggttgctatccccacgcatacgaaatgacatacgaaatctctatgcagtagttcgtatcgccgatgagattgtcgacggcactgcacatgccgctggttgctcaactgccaaaatcgaagagattctcgatgcctatgaaattgcggttcttgcagcaccacaacaacgcttcaacacagatcttgttttacaagcttatggtgaaactgcccgacgctgtgatttcgaacaagagcatgtaatagccttctttgcatcaatgcgtaaggacctcaaagctaatacacacgacccagatagcttcacaacgtatgtctatggctccgcggaagttataggcctgctttgtctcagcgttttcaaccaaggtagaacgattagcaaaaaacggctagagattatgcaaaacggagcccgctcattgggagcggcattccagaaaattaactttctccgtgacttggcagaagatcagcaaaatttgggccgattttatttccccaaaaccagccaaggaactcttactaaagaacaaaaagaagatctcatcgctgatatccgtcaagacctagcaattgcccacgatgcatttccagaaataccagtgcaggctcgcatcggagtgatctctgcttatttgctctttcaaaaactcactgaccgaattgaggctactcctaccgccgatttattgcgggagcgaatcagagttccacttcatatcaaactctctacactcgctagagccacgatgaaaggtctatctatgagcatctacagaaagaattcgtga

SEQ ID NO: 4 - protein, 304 aa, Corynebacterium glutamicum
MTHQNSPLFLKSALRLYNRASFKASHKVIEEYSTSFSLSTWLLSPRIRNDIRNLYAVVRIADEIVDGTAHAAGCSTAKIEEILDAYEIAVLAAPQQRFNTDLVLQAYGETARRCDFEQEHVIAFFASMRKDLKANTHDPDSFTTYVYGSAEVIGLLCLSVFNQGRTISKKRLEIMQNGARSLGAAFQKINFLRDLAEDQQNLGRFYFPKTSQGTLTKEQKEDLIADIRQDLAIAHDAFPEIPVQARIGVISAYLLFQKLTDRIEATPTADLLRERIRVPLHIKLSTLARATMKGLSMSIYRKNS

SEQ ID NO: 5 - DNA, 1647 bp, Corynebacterium glutamicum
  source 1..1647: mol_type = genomic DNA
atgaaggtctcgactaaaactccacgctcctcaggtaccgccgtagtcataggcgcaggtgttgctggtttagccacttctgcacttttagcacgtgatggctggcaagtaactgttttggaaaaaaatactgatgtcggtggccgagctggatcgcttgaaatatcaggctttcctggctttcgatgggataccggaccttcttggtacctcatgcccgaggcctttgaccatttcttcgcactttttggtgcatgtacttctgattatctcgatttggtagaattaacgcctggttatcgagttttttctggcacacatgacgctgtcgatgtccccactgggcgtgaagaagcaattgcgctattcgaatccatcgaacccggcgcgggtgcaaaactaggaaattatcttgatagcgcggcagacgcctatgacattgccattgatagattcctttataataatttctccacgttaggcccgctgcttcaccgggatgtactgacccgagctggccgactgttttctctactgacccgttctttacaaaagtacgtaaatagtcaattcagtagcccggtgttgcgccagatcctaacctatccagcagtcttcctgtcttcccgacccactactaccccatcgatgtaccacttgatgagtcataccgatttggtgcagggagtgaaataccctataggtggttttactgcagtggttaacgctctgcatcagttagcgctggaaaacggggttgagtttcaactcgattctgaggtcatttccatcaacactgcttcatcgaggggcaacacaagcgccacaggtgtgagcttgcttcacaacagaaaagtgcaaaatctagatgcggatcttgtggtttcagcaggcgacctacaccatacagaaaataatctgcttccccgggaacttcgaacctatcccgaacgatattggtccaatcgcaatcctggaattggagcggtattaatcctcctgggcgtaaaaggagagttaccccagctcgaccatcacaaccttttcttcagtgaagattggacagatgattttgctgtagttttcgacgggcctcaacttacccgcccccacaatgcatcaaattccatttatgtctccaagccttcaacgtccgaagacggcgttgcacctgctggatacgaaaacctttttgttttaattccgaccaaggcctctagcagcatcggccacggtgatgcgtatatgcagtcggcttcagcatccgtggaaacaatcgcgtcacatgcaatcaatcaaattgctacgcaagccggcatccctgacctcactgaccgaattgtggtcaaacgcaccattggccctgcggattttgagcaccgctaccattcatgggtaggcagtgcgctgggtccagcacataccctcagacagtccgctttcttaagagggcgcaatagctcccgcaaggtcaataacctcttctattccggtgccaccaccgtcccgggtgtaggaatacccatgtgtttaatttctgccgagaatattattaagcgtttacatgccgataccagtgcaggaccactgcccgaaccattgccgcctaaaacgacaccatctcaaaagacctcatacgatcattaa

SEQ ID NO: 6 - protein, 548 aa, Corynebacterium glutamicum
MKVSTKTPRSSGTAVVIGAGVAGLATSALLARDGWQVTVLEKNTDVGGRAGSLEISGFPGFRWDTGPSWYLMPEAFDHFFALFGACTSDYLDLVELTPGYRVFSGTHDAVDVPTGREEAIALFESIEPGAGAKLGNYLDSAADAYDIAIDRFLYNNFSTLGPLLHRDVLTRAGRLFSLLTRSLQKYVNSQFSSPVLRQILTYPAVFLSSRPTTTPSMYHLMSHTDLVQGVKYPIGGFTAVVNALHQLALENGVEFQLDSEVISINTASSRGNTSATGVSLLHNRKVQNLDADLVVSAGDLHHTENNLLPRELRTYPERYWSNRNPGIGAVLILLGVKGELPQLDHHNLFFSEDWTDDFAVVFDGPQLTRPHNASNSIYVSKPSTSEDGVAPAGYENLFVLIPTKASSSIGHGDAYMQSASASVETIASHAINQIATQAGIPDLTDRIVVKRTIGPADFEHRYHSWVGSALGPAHTLRQSAFLRGRNSSRKVNNLFYSGATTVPGVGIPMCLISAENIIKRLHADTSAGPLPEPLPPKTTPSQKTSYDH

SEQ ID NO: 7 - DNA, 879 bp, Corynebacterium glutamicum
  source 1..879: mol_type = genomic DNA
gtgaaggaggcgagtgtggctgatcagcaagattttttgggccgttttgatgcgatgagctcaaaggcgacggccacggtaatcgcccattattcctccagttttactctggcatcgaagctgttgtcgccgaaaattcgtcgcgatattgaggcattgtacgcaatggtgcgagtggccgatgaggttgtggacggcgctgctgctgccgcggggtgtgcgccggacgccgttgcggagattttggacaattacgaacgccaggttctgctcagtttgtccgttccttttcataccgatccagtgatccatgcgtttggcaataccgcccgcaaatgtggttttgagcaggctcacatcgtggcgttttttgattccatgcgccgcgatctctcccaaacctcctatgatccgactcagttggatgagtacatttacggctccgctgaggtcatcgggttgatgtgtttgaaaattttcctccaagattccactgccagcccgcaggatcgggccacgatggaacacggcgccaggcgtttgggtgcggcatttcaaaaggtaaatttcctgcgagatctagctgaagaccgcgaaggcctaggccgttcttatttgccggtattcaccgaagaaatgcgcgatgagatcgttactgatatccgagaggatttggatgccgcccggctgagcattccgctgctgccatttggcgcgcgaaccggtgtgcgcgccgcgaccgatctctacggttgcctcgtggacaacctggaatccgcgtccctcgaagacttaaaaaacgggcggattcgggtgccgtctatgaaaaaagccagcctggcaaccaaagcaatgtggaaagaagtgtttcaaaaatga

SEQ ID NO: 8 - protein, 292 aa, Corynebacterium glutamicum
MKEASVADQQDFLGRFDAMSSKATATVIAHYSSSFTLASKLLSPKIRRDIEALYAMVRVADEVVDGAAAAAGCAPDAVAEILDNYERQVLLSLSVPFHTDPVIHAFGNTARKCGFEQAHIVAFFDSMRRDLSQTSYDPTQLDEYIYGSAEVIGLMCLKIFLQDSTASPQDRATMEHGARRLGAAFQKVNFLRDLAEDREGLGRSYLPVFTEEMRDEIVTDIREDLDAARLSIPLLPFGARTGVRAATDLYGCLVDNLESASLEDLKNGRIRVPSMKKASLATKAMWKEVFQK

SEQ ID NO: 9 - DNA, 1209 bp, Corynebacterium glutamicum
  source 1..1209: mol_type = genomic DNA
gtggaaagaagtgtttcaaaaatgacaaaagcagtggtcatcggcgggggactagcaggactagccaccaccgcactgctcttacgcgaaggatatgaagtccacctcgtcgaacaaaacgagcacctcggcggccgcgccgggaccttcgaactcgacggcttccgctgggacaccggccccagctggtacctcatgcccgacgccatgtcccacttctttaagctctgcggcacctccatcgacgaccacctcgacctcgtgccacttgaacccgcctaccgcgtcatcgacgaccacggcgaattcatcgacgtcacctccgacatcgatgcgatggccgagcttttcgaatcccgcgaacccggcgccggcgccaaactgcgcacctatatcgactccgccacacaggtctacaacctggccatcgacggcttcctctacaccaacttcaccaacttcatcccatacttaagccccggcatgctgcgccttttacccaaacttctagcaagcctgtcgacctcgctaaaagtcaaggtcaacacccaattccgcgatacaaaactgcgccaaatcttaagctaccccgcagttttcctctcctcagacccttcgcacaccccggcgctctatcacctcatgagccacaccgacctcgtccaaggcgtctcctatccccgaggcggcttcaccgccttcatcaaggcactaatttcgcttatcgacgacgccgtcctccacctcggcacccccgtcagcgcaatcaccacccaaggccgaaacgccacaggcgtccaagtcggctcagagttcatcgaagccgatatcgtgatcagctgcgctgatcagcaccacaccgaaacccaactcctacctgcttcgttgtgcgcgaagccggagacgagctggaagaacaaacaacccggcctcagtactgtgctggttttggcaggcgtgaagggggagcacaccctgctttttcctccgactgggacgaagatttccgcaaagttttcgacggctccaccccagaattcccggcttcagaatccatctagatctccaagacctccgcaacagattccgatgccgcacccgaaggccacgagaacctcttcatcctggtcccagtacccgccgatgtctccattggtcacgggtccgcttacggagaagaatctgacatggtgggccggatcgcaatag

SEQ ID NO: 10 - protein, 402 aa, Corynebacterium glutamicum
MERSVSKMTKAVVIGGGLAGLATTALLLREGYEVHLVEQNEHLGGRAGTFELDGFRWDTGPSWYLMPDAMSHFFKLCGTSIDDHLDLVPLEPAYRVIDDHGEFIDVTSDIDAMAELFESREPGAGAKLRTYIDSATQVYNLAIDGFLYTNFTNFIPYLSPGMLRLLPKLLASLSTSLKVKVNTQFRDTKLRQILSYPAVFLSSDPSHTPALYHLMSHTDLVQGVSYPRGGFTAFIKALISLIDDAVLHLGTPVSAITTQGRNATGVQVGSEFIEADIVISCADQHHTETQLLPASLCAKPETSWKNKQPGLSTVLVLAGVKGEHTLLFPPTGTKISAKFSTAPPQNSRLQNPSRSPRPPQQIPMPHPKATRTSSSWSQYPPMSPLVTGPLTEKNLTWWAGSQ

SEQ ID NO: 11 - DNA, 330 bp, Corynebacterium glutamicum
  source 1..330: mol_type = genomic DNA
atggtgggccggatcgcaatagcagcagtggctcaaattgggcgatgggctggcattgatggtttggaaagccgcattgttgtgcagcgcaccatcggccctgccgacttcgcagaccgatacaactcctggagcggcgggtccattggcccctcacacaccctggcacaatcggcgttctttaggggttctaacaaatcccgcaaagtagatggcctgtatgacgcaggtgacaccacagttccaggggtgggcgtatctatgtgtttgatctctgcagaaaacgtgctcaagcgtctccgcggggacaacagtgtggatcggacttaa

SEQ ID NO: 12 - protein, 109 aa, Corynebacterium glutamicum
MVGRIAIAAVAQIGRWAGIDGLESRIVVQRTIGPADFADRYNSWSGGSIGPSHTLAQSAFFRGSNKSRKVDGLYDAGDTTVPGVGVSMCLISAENVLKRLRGDNSVDRT

SEQ ID NO: 13 - DNA, 30 bp, synthetic construct
  source 1..30: mol_type = other DNA
tgattacgccgcatcgcctctccacgagtg

SEQ ID NO: 14 - DNA, 20 bp, synthetic construct
  source 1..20: mol_type = other DNA
gcatcgcctctccacgagtg

SEQ ID NO: 15 - DNA, 20 bp, synthetic construct
  source 1..20: mol_type = other DNA
tcgttgtatatggcgcttta

SEQ ID NO: 16 - DNA, 20 bp, synthetic construct
  source 1..20: mol_type = other DNA
aaattcccaatcgttgtata

SEQ ID NO: 17 - DNA, 30 bp, synthetic construct
  source 1..30: mol_type = other DNA
ttgggaatttatgaaggtctcgactaaaac

SEQ ID NO: 18 - DNA, 20 bp, synthetic construct
  source 1..20: mol_type = other DNA
atgaaggtctcgactaaaac

SEQ ID NO: 19 - DNA, 20 bp, synthetic construct
  source 1..20: mol_type = other DNA
ggaagacaggaagactgctg

SEQ ID NO: 20 - DNA, 20 bp, synthetic construct
  source 1..20: mol_type = other DNA
tagtgggtcgggaagacagg

SEQ ID NO: 21 - DNA, 30 bp, synthetic construct
  source 1..30: mol_type = other DNA
tgattacgccgcttatggtgaaactgcccg

SEQ ID NO: 22 - DNA, 20 bp, synthetic construct
  source 1..20: mol_type = other DNA
gcttatggtgaaactgcccg

SEQ ID NO: 23 - DNA, 20 bp, synthetic construct
  source 1..20: mol_type = other DNA
tttctgtagatgctcataga

SEQ ID NO: 24 - DNA, 20 bp, synthetic construct
  source 1..20: mol_type = other DNA
tcacgaattctttctgtaga

SEQ ID NO: 25 - DNA, 30 bp, synthetic construct
  source 1..30: mol_type = other DNA
gaattcgtgaattttgatccctatcatcga

SEQ ID NO: 26 - DNA, 20 bp, synthetic construct
  source 1..20: mol_type = other DNA
attttgatccctatcatcga

SEQ ID NO: 27 - DNA, 20 bp, synthetic construct
  source 1..20: mol_type = other DNA
aggttatcaaatatgatagt

SEQ ID NO: 28 - DNA, 20 bp, synthetic construct
  source 1..20: mol_type = other DNA
ccaaaccatgaggttatcaa

SEQ ID NO: 29 - DNA, 30 bp, synthetic construct
  source 1..30: mol_type = other DNA
tgattacgccggggaccgaccatcatccac

SEQ ID NO: 30 - DNA, 20 bp, synthetic construct
  source 1..20: mol_type = other DNA
ggggaccgaccatcatccac

SEQ ID NO: 31 - DNA, 20 bp, synthetic construct
  source 1..20: mol_type = other DNA
accgcgagaaatccagacaa

SEQ ID NO: 32 - DNA, 20 bp, synthetic construct
  source 1..20: mol_type = other DNA
aggaaactttaccgcgagaa

SEQ ID NO: 33 - DNA, 30 bp, synthetic construct
  source 1..30: mol_type = other DNA
aaagtttcctgtggaaagaagtgtttcaaa

SEQ ID NO: 34 - DNA, 20 bp, synthetic construct
  source 1..20: mol_type = other DNA
gtggaaagaagtgtttcaaa

SEQ ID NO: 35 - DNA, 20 bp, synthetic construct
  source 1..20: mol_type = other DNA
gggtagcttaagatttggcg

SEQ ID NO: 36 - DNA, 20 bp, synthetic construct
  source 1..20: mol_type = other DNA
gaaaactgcggggtagctta

SEQ ID NO: 37 - DNA, 30 bp, synthetic construct
  source 1..30: mol_type = other DNA
tgattacgcctcagtttgtccgttcctttt

SEQ ID NO: 38 - DNA, 19 bp, synthetic construct
  source 1..19: mol_type = other DNA
tcagtttgtccgttccttt

SEQ ID NO: 39 - DNA, 20 bp, synthetic construct
  source 1..20: mol_type = other DNA
aacacttctttccacattgc

SEQ ID NO: 40 - DNA, 20 bp, synthetic construct
  source 1..20: mol_type = other DNA
tcatttttgaaacacttctt

SEQ ID NO: 41 - DNA, 30 bp, synthetic construct
  source 1..30: mol_type = other DNA
tcaaaaatgacctggagcggcgggtccatt

SEQ ID NO: 42 - DNA, 20 bp, synthetic construct
  source 1..20: mol_type = other DNA
cctggagcggcgggtccatt

SEQ ID NO: 43 - DNA, 20 bp, synthetic construct
  source 1..20: mol_type = other DNA
gaatgttggtgaaccatttg

SEQ ID NO: 44 - DNA, 20 bp, synthetic construct
  source 1..20: mol_type = other DNA
tcggctgcatgaatgttggt